European Patent Application EP 4 740 954 A2, published May 13, 2026. Title: COMPOSITIONS AND METHODS FOR TREATMENT OF NETHERTON SYNDROME WITH LEKTI EXPRESSING RECOMBINANT MICROBES. Applicant: AZITRA, INC. The sequence listing filed with the application follows.

SEQUENCE LISTING (125 sequences)

SEQ ID NO: 1-8 - skipped (8 entries)

SEQ ID NO: 9 - protein, 25 aa, unidentified
  REGION 1..25: note = Description of Unknown: Secretion peptide
MKKLAFAITAASGAAAVLSHHDAEA

SEQ ID NO: 10 - protein, 30 aa, unidentified
  REGION 1..30: note = Description of Unknown: Secretion peptide
WLDNRAFSKKFVPVVMATSVALFFLNLAFA

SEQ ID NO: 11 - protein, 29 aa, unidentified
  REGION 1..29: note = Description of Unknown: Secretion peptide
MAKKFNYKLPSMVALTLFGTAFTAHQANA

SEQ ID NO: 12 - protein, 27 aa, unidentified
  REGION 1..27: note = Description of Unknown: Secretion peptide
MKKRFLSICTMTIAALATTTMVNTSYA

SEQ ID NO: 13 - protein, 30 aa, unidentified
  REGION 1..30: note = Description of Unknown: Secretion peptide
NLKKQSKLILIFICIFTFFIMIIQSQFLMG

SEQ ID NO: 14 - protein, 26 aa, unidentified
  REGION 1..26: note = Description of Unknown: Secretion peptide
MKIFKLTSLTLAALTLAFPFSHVAQA

SEQ ID NO: 15 - protein, 27 aa, unidentified
  REGION 1..27: note = Description of Unknown: Secretion peptide
MKKTVIASTLAVSLGIAGYGLSGHEAH

SEQ ID NO: 16 - protein, 27 aa, unidentified
  REGION 1..27: note = Description of Unknown: Secretion peptide
MKKNKFLVYLLSTALITPTFATQTAFA

SEQ ID NO: 17 - protein, 35 aa, unidentified
  REGION 1..35: note = Description of Unknown: Secretion peptide
MKTRQNKYSIRKFSVGASSILIAALLFMGGGSAQA

SEQ ID NO: 18 - protein, 37 aa, unidentified
  REGION 1..37: note = Description of Unknown: Secretion peptide
MKNNNETRRFSIRKYTVGVVSIITGITIFVSGQHAQA

SEQ ID NO: 19 - protein, 30 aa, unidentified
  REGION 1..30: note = Description of Unknown: Secretion peptide
MKKKLSYMITIMLAFTLSLALGLFFNSAHA

SEQ ID NO: 20 - protein, 45 aa, Staphylococcus epidermidis
MKKRRQGPINKRVDFLSNKVNKYSIRKFTVGTASILVGATLMFGA

SEQ ID NO: 21 - protein, 27 aa, Staphylococcus epidermidis
MKKRFLSICTMTIAALATTTMVNTSYA

SEQ ID NO: 22 - protein, 29 aa, Staphylococcus epidermidis
MAKKFNYKLPSMVALTLFGTAFTAHQANA

SEQ ID NO: 23 - protein, 50 aa, Staphylococcus epidermidis
MIKKNNLLTKKKPIANKSNKYAIRKFTVGTASIVIGAALLFGLGHNEAKA

SEQ ID NO: 24 - protein, 30 aa, Staphylococcus epidermidis
MKPFKLIFISALMILIMTNATPISHLNAQA

SEQ ID NO: 25 - protein, 35 aa, Staphylococcus epidermidis; identical to SEQ ID NO: 17

SEQ ID NO: 26 - protein, 23 aa, Staphylococcus epidermidis
MNKFKFFIVFLILSLVFLQNEYA

SEQ ID NO: 27 - protein, 51 aa, Staphylococcus epidermidis
MINKKNNLLTKKKPIANKSNKYAIRKFTVGTASIVIGATLLFGLGHNEAKA

SEQ ID NO: 28 - protein, 26 aa, Staphylococcus epidermidis
MKKIATATIATAGIATFAFAHHDAQA

SEQ ID NO: 29 - protein, 28 aa, Staphylococcus epidermidis
MKNFSKFALTSIAALTVASPLVNTEVDA

SEQ ID NO: 30 - protein, 37 aa, Staphylococcus epidermidis; identical to SEQ ID NO: 18

SEQ ID NO: 31 - protein, 19 aa, Staphylococcus epidermidis
MRYLKRITIYISLLILVSG

SEQ ID NO: 32 - protein, 20 aa, Staphylococcus epidermidis
MKLMNKIIVPVTASALLLGA

SEQ ID NO: 33 - protein, 40 aa, Staphylococcus epidermidis
MKKIDSWLTKHGLKNRLTLVVIVIFIIFLILLFMFVNLSD

SEQ ID NO: 34 - protein, 19 aa, Staphylococcus epidermidis
MKKKALLPLFLGIMIFLAG

SEQ ID NO: 35 - protein, 28 aa, Staphylococcus epidermidis
MKKTVIASTLAVSLGIAGYGLSGHEAHA

SEQ ID NO: 36 - protein, 19 aa, Staphylococcus epidermidis
MSKFKSLLLLFGTLILLSG

SEQ ID NO: 37 - protein, 27 aa, Staphylococcus epidermidis
MKKTLVASSLAIGLGVVAGNAGHDAHA

SEQ ID NO: 38 - protein, 29 aa, Staphylococcus epidermidis
MAKKFNYKLPSMVALTLFGTAFTAHQANA

SEQ ID NO: 39 - protein, 30 aa, Staphylococcus epidermidis; identical to SEQ ID NO: 19

SEQ ID NO: 40 - protein, 18 aa, Staphylococcus epidermidis
MHKRLFITLLGFIILLAG

SEQ ID NO: 41 - protein, 19 aa, Staphylococcus epidermidis
MRYLKRITIYISLLILVSG

SEQ ID NO: 42 - protein, 25 aa, Staphylococcus epidermidis
MQKKYITAIIGTTALSALASTHAQA

SEQ ID NO: 43 - protein, 22 aa, Staphylococcus epidermidis
MKHSSKIIVFVSFLILTIFIGG

SEQ ID NO: 44 - protein, 20 aa, Staphylococcus epidermidis
MKKWQLVGTTVLGASVLLGA

SEQ ID NO: 45 - protein, 52 aa, Staphylococcus epidermidis
MGKRRQGPINKKVDFLPNKLNKYSIRKFTVGTASILLGSTLIFGSSSHEAKA

SEQ ID NO: 46 - protein, 26 aa, Staphylococcus epidermidis
MKKIATATIATAGIATFAFAHHDAQA

SEQ ID NO: 47 - protein, 45 aa, Staphylococcus epidermidis; identical to SEQ ID NO: 20

SEQ ID NO: 48 - protein, 27 aa, Staphylococcus epidermidis
MKKRFLSICTMTIAALATTTMVNTSYA

SEQ ID NO: 49 - protein, 35 aa, Staphylococcus epidermidis; identical to SEQ ID NO: 17

SEQ ID NO: 50 - protein, 28 aa, Staphylococcus epidermidis
MKNFSKFALTSIAALTVASPLVNTEVDA

SEQ ID NO: 51 - protein, 17 aa, Staphylococcus epidermidis
MKKVLASATILSLMLVG

SEQ ID NO: 52 - protein, 22 aa, Staphylococcus epidermidis
MKYYGKCISYISILILTFFIGG

SEQ ID NO: 53 - protein, 22 aa, Staphylococcus epidermidis
MKHSSKIIVFVSFLILTIFIGG

SEQ ID NO: 54 - protein, 30 aa, Staphylococcus epidermidis; identical to SEQ ID NO: 24

SEQ ID NO: 55 - protein, 19 aa, Staphylococcus epidermidis
MSKFKSLLLLFGTLILLSG

SEQ ID NO: 56 - protein, 27 aa, Staphylococcus epidermidis
MKKTLVASSLAIGLGVVAGNAGHDAHA

SEQ ID NO: 57 - protein, 19 aa, Staphylococcus epidermidis
MHYLKKVTIYISLLILVSG

SEQ ID NO: 58 - protein, 25 aa, Staphylococcus epidermidis
MQKKYITAIIGTTALSALASTHAQA

SEQ ID NO: 59 - protein, 22 aa, Staphylococcus epidermidis
MKHSKKLLLCISFLLITFFIGG

SEQ ID NO: 60 - protein, 26 aa, Staphylococcus epidermidis
MKKIATATIATAGIATFAFAHHDAQA

SEQ ID NO: 61 - protein, 19 aa, Staphylococcus epidermidis
MRYLKKVTIYISLLILVSG

SEQ ID NO: 62 - protein, 27 aa, Staphylococcus epidermidis
MKKRFLSICTMTIAALATTTMVNTSYA

SEQ ID NO: 63 - protein, 20 aa, Staphylococcus epidermidis
MKKWQLVGTTVLGASVLLGA

SEQ ID NO: 64 - protein, 29 aa, Staphylococcus epidermidis
MAKKFNYKLPSMVALTLFGTAFTAHQANA

SEQ ID NO: 65 - protein, 30 aa, Staphylococcus epidermidis; identical to SEQ ID NO: 19

SEQ ID NO: 66 - protein, 18 aa, Staphylococcus epidermidis
MHKRLFITLLGFIILLAG

SEQ ID NO: 67 - protein, 22 aa, Staphylococcus epidermidis
MRYLKKVTIYISLLILTIFIGG

SEQ ID NO: 68 - protein, 17 aa, Staphylococcus epidermidis
MKKVLASATILSLMLVG

SEQ ID NO: 69 - protein, 22 aa, Staphylococcus epidermidis
MKHSKKLLLCISFLLITVFISG

SEQ ID NO: 70 - protein, 22 aa, Staphylococcus epidermidis
MKHSKKLLLCISFLLITFFISG

SEQ ID NO: 71 - protein, 28 aa, Staphylococcus epidermidis
MKKTVIASTLAVSLGIAGYGLSGHEAHA

SEQ ID NO: 72 - protein, 22 aa, Staphylococcus epidermidis
MKHSKKLLLCISFLLITIFISG

SEQ ID NO: 73 - protein, 40 aa, Staphylococcus epidermidis; identical to SEQ ID NO: 33

SEQ ID NO: 74 - protein, 19 aa, Staphylococcus epidermidis
MKKKALLPLFLGIMIFLAG

SEQ ID NO: 75 - protein, 20 aa, Staphylococcus epidermidis
MKLMNKIIVPVTASALLLGA

SEQ ID NO: 76 - protein, 35 aa, Staphylococcus epidermidis; identical to SEQ ID NO: 17

SEQ ID NO: 77 - protein, 13 aa, unidentified
  REGION 1..13: note = Description of Unknown: Cell penetrating peptide
GRKKRRQRRRPPQ

SEQ ID NO: 78 - protein, 27 aa, unidentified
  REGION 1..27: note = Description of Unknown: Cell penetrating peptide
GWTLNSAGYLLGKINLKALAALAKKIL

SEQ ID NO: 79 - protein, 18 aa, unidentified
  REGION 1..18: note = Description of Unknown: Cell penetrating peptide
KLALKLALKALKAALKLA

SEQ ID NO: 80 - protein, 30 aa, unidentified
  REGION 1..30: note = Description of Unknown: Cell penetrating peptide
WEAKLAKALAKALAKHLAKALAKALKACEA

SEQ ID NO: 81 - protein, 21 aa, unidentified
  REGION 1..21: note = Description of Unknown: Cell penetrating peptide
KETWWETWWTEWSQPKKKRKV

SEQ ID NO: 82 - protein, 9 aa, unidentified
  REGION 1..9: note = Description of Unknown: Cell penetrating peptide
RRRRRRRRR

SEQ ID NO: 83 - protein, 24 aa, unidentified
  REGION 1..24: note = Description of Unknown: Cell penetrating peptide
LGTYTQDFNKFHTFPQTAIGVGAP

SEQ ID NO: 84 - protein, 15 aa, unidentified
  REGION 1..15: note = Description of Unknown: Cell penetrating peptide
RQIKWFQNRRMKWKK

SEQ ID NO: 85 - protein, 11 aa, unidentified
  REGION 1..11: note = Description of Unknown: Cell penetrating peptide
YGRKKRRQRRR

SEQ ID NO: 86 - protein, 18 aa, unidentified
  REGION 1..18: note = Description of Unknown: Cell penetrating peptide
RGGRLSYSRRRFSTSTGR

SEQ ID NO: 87 - protein, 10 aa, unidentified
  REGION 1..10: note = Description of Unknown: Cell penetrating peptide
RRLSYSRRRF

SEQ ID NO: 88 - protein, 12 aa, unidentified
  REGION 1..12: note = Description of Unknown: Cell penetrating peptide
PIRRRKKLRRLK

SEQ ID NO: 89 - protein, 12 aa, unidentified
  REGION 1..12: note = Description of Unknown: Cell penetrating peptide
RRQRRTSKLMKR

SEQ ID NO: 90 - protein, 15 aa, unidentified
  REGION 1..15: note = Description of Unknown: Cell penetrating peptide
RRRRNRTRRNRRRVR

SEQ ID NO: 91 - protein, 19 aa, unidentified
  REGION 1..19: note = Description of Unknown: Cell penetrating peptide
KMTRAQRRAAARRNRWTAR

SEQ ID NO: 92 - protein, 13 aa, unidentified
  REGION 1..13: note = Description of Unknown: Cell penetrating peptide
TRRQRTRRARRNR

SEQ ID NO: 93 - protein, 13 aa, unidentified
  REGION 1..13: note = Description of Unknown: Cell penetrating peptide
GRKKRRQRRRPPQ

SEQ ID NO: 94 - protein, 13 aa, unidentified
  REGION 1..13: note = Description of Unknown: Cell penetrating peptide
GRRRRRRRRRPPQ

SEQ ID NO: 95 - protein, 27 aa, unidentified
  REGION 1..27: note = Description of Unknown: Cell penetrating peptide
GWTLNSAGYLLGKINLKALAALAKKIL

SEQ ID NO: 96 - protein, 17 aa, unidentified
  REGION 1..17: note = Description of Unknown: Cell penetrating peptide
KLALKLALKLALALKLA

SEQ ID NO: 97 - protein, 27 aa, unidentified
  REGION 1..27: note = Description of Unknown: Cell penetrating peptide
MGLGLHLLVLAAALQGAWSQPKKKRKV

SEQ ID NO: 98 - protein, 27 aa, unidentified
  REGION 1..27: note = Description of Unknown: Cell penetrating peptide
GALFLGWLGAAGSTMGAWSQPKKKRKV

SEQ ID NO: 99 - protein, 27 aa, unidentified
  REGION 1..27: note = Description of Unknown: Cell penetrating peptide
GALFLGFLGAAGSTMGAWSQPKKKRKV

SEQ ID NO: 100 - protein, 27 aa, unidentified
  REGION 1..27: note = Description of Unknown: Cell penetrating peptide
GALFLGFLGAAGSTMGAWSQPKSKRKV

SEQ ID NO: 101 - protein, 21 aa, unidentified
  REGION 1..21: note = Description of Unknown: Cell penetrating peptide
KETWWETWWTEWSQPKKKRKV

SEQ ID NO: 102 - protein, 21 aa, unidentified
  REGION 1..21: note = Description of Unknown: Cell penetrating peptide
KETWFETWFTEWSQPKKKRKV

SEQ ID NO: 103 - protein, 1064 aa, unidentified
  REGION 1..1064: note = Description of Unknown: sequence
MKIATVSVLLPLALCLIQDAASKNEDQEMCHEFQAFMKNGKLFCPQDKKFFQSLDGIMFINKCATCKMILEKEAKSQKRARHLARAPKATAPTELNCDDFKKGERDGDFICPDYYEAVCGTDGKTYDNRCALCAENAKTGSQIGVKSEGECKSSNPEQDVCSAFRPFVRDGRLGCTRENDPVLGPDGKTHGNKCAMCAELFLKEAENAKREGETRIRRNAEKDFCKEYEKQVRNGRLFCTRESDPVRGPDGRMHGNKCALCAEIFKQRFSEENSKTDQNLGKAEEKTKVKREIVKLCSQYQNQAKNGILFCTRENDPIRGPDGKMHGNLCSMCQAYFQAENEEKKKAEARARNKRESGKATSYAELCSEYRKLVRNGKLACTRENDPIQGPDGKVHGNTCSMCEVFFQAEEEEKKKKEGKSRNKRQSKSTASFEELCSEYRKSRKNGRLFCTRENDPIQGPDGKMHGNTCSMCEAFFQQEERARAKAKREAAKEICSEFRDQVRNGTLICTREHNPVRGPDGKMHGNKCAMCASVFKLEEEEKKNDKEEKGKVEAEKVKREAVQELCSEYRHYVRNGRLPCTRENDPIEGLDGKIHGNTCSMCEAFFQQEAKEKERAEPRAKVKREAEKETCDEFRRLLQNGKLFCTRENDPVRGPDGKTHGNKCAMCKAVFQKENEERKRKEEEDQRNAAGHGSSGGGGGNTQDECAEYREQMKNGRLSCTRESDPVRDADGKSYNNQCTMCKAKLEREAERKNEYSRSRSNGTGSESGKDTCDEFRSQMKNGKLICTRESDPVRGPDGKTHGNKCTMCKEKLEREAAEKKKKEDEDRSNTGERSNTGERSNDKEDLCREFRSMQRNGKLICTRENNPVRGPYGKMHINKCAMCQSIFDREANERKKKDEEKSSSKPSNNAKDECSEFRNYIRNNELICPRENDPVHGADGKFYTNKCYMCRAVFLTEALERAKLQEKPSHVRASQEEDSPDSFSSLDSEMCKDYRVLPRIGYLCPKDLKPVCGDDGQTYNNPCMLCHENLIRQTNTHIRSTGKCEESSTPGTTAASMPPSDE

SEQ ID NO: 104 - protein, 55 aa, unidentified
  REGION 1..55: note = Description of Unknown: sequence
KNEDQEMCHEFQAFMKNGKLFCPQDKKFFQSLDGIMFINKCATCKMILEKEAKSQ

SEQ ID NO: 105 - protein, 63 aa, unidentified
  REGION 1..63: note = Description of Unknown: sequence
APTELNCDDFKKGERDGDFICPDYYEAVCGTDGKTYDNRCALCAENAKTGSQIGVKSEGECKS

SEQ ID NO: 106 - protein, 62 aa, unidentified
  REGION 1..62: note = Description of Unknown: sequence
NPEQDVCSAFRPFVRDGRLGCTRENDPVLGPDGKTHGNKCAMCAELFLKEAENAKREGETRI

SEQ ID NO: 107 - protein, 67 aa, unidentified
  REGION 1..67: note = Description of Unknown: sequence
NAEKDFCKEYEKQVRNGRLFCTRESDPVRGPDGRMHGNKCALCAEIFKQRFSEENSKTDQNLGKAEE

SEQ ID NO: 108 - protein, 62 aa, unidentified
  REGION 1..62: note = Description of Unknown: sequence
REIVKLCSQYQNQAKNGILFCTRENDPIRGPDGKMHGNLCSMCQAYFQAENEEKKKAEARAR

SEQ ID NO: 109 - protein, 68 aa, unidentified
  REGION 1..68: note = Description of Unknown: sequence
ESGKATSYAELCSEYRKLVRNGKLACTRENDPIQGPDGKVHGNTCSMCEVFFQAEEEEKKKKEGKSRN

SEQ ID NO: 110 - protein, 59 aa, unidentified
  REGION 1..59: note = Description of Unknown: sequence
ASFEELCSEYRKSRKNGRLFCTRENDPIQGPDGKMHGNTCSMCEAFFQQEERARAKAKR

SEQ ID NO: 111 - protein, 62 aa, unidentified
  REGION 1..62: note = Description of Unknown: sequence
EAAKEICSEFRDQVRNGTLICTREHNPVRGPDGKMHGNKCAMCASVFKLEEEEKKNDKEEKG

SEQ ID NO: 112 - protein, 62 aa, unidentified
  REGION 1..62: note = Description of Unknown: sequence
EAVQELCSEYRHYVRNGRLPCTRENDPIEGLDGKIHGNTCSMCEAFFQQEAKEKERAEPRAK

SEQ ID NO: 113 - protein, 63 aa, unidentified
  REGION 1..63: note = Description of Unknown: sequence
EAEKETCDEFRRLLQNGKLFCTRENDPVRGPDGKTHGNKCAMCKAVFQKENEERKRKEEEDQR

SEQ ID NO: 114 - protein, 57 aa, unidentified
  REGION 1..57: note = Description of Unknown: sequence
GNTQDECAEYREQMKNGRLSCTRESDPVRDADGKSYNNQCTMCKAKLEREAERKNEY

SEQ ID NO: 115 - protein, 63 aa, unidentified
  REGION 1..63: note = Description of Unknown: sequence
ESGKDTCDEFRSQMKNGKLICTRESDPVRGPDGKTHGNKCTMCKEKLEREAAEKKKKEDEDRS

SEQ ID NO: 116 - protein, 63 aa, unidentified
  REGION 1..63: note = Description of Unknown: sequence
NDKEDLCREFRSMQRNGKLICTRENNPVRGPYGKMHINKCAMCQSIFDREANERKKKDEEKSS

SEQ ID NO: 117 - protein, 62 aa, unidentified
  REGION 1..62: note = Description of Unknown: sequence
NNAKDECSEFRNYIRNNELICPRENDPVHGADGKFYTNKCYMCRAVFLTEALERAKLQEKPS

SEQ ID NO: 118 - protein, 62 aa, unidentified
  REGION 1..62: note = Description of Unknown: sequence
SLDSEMCKDYRVLPRIGYLCPKDLKPVCGDDGQTYNNPCMLCHENLIRQTNTHIRSTGKCEE

SEQ ID NO: 119 - DNA, 3192 bp, synthetic construct
  misc_feature 1..3192: note = Description of Artificial Sequence: Synthetic polynucleotide
  source 1..3192: mol_type = other DNA
atgaagatagccacagtgtcagtgcttctgcccttggctctttgcctcatacaagatgctgccagtaagaatgaagatcaggaaatgtgccatgaatttcaggcatttatgaaaaatggaaaactgttctgtccccaggataagaaattttttcaaagtcttgatggaataatgttcatcaataaatgtgccacgtgcaaaatgatactggaaaaagaagcaaaatcacagaagagggccaggcatttagcaagagctcccaaggctactgccccaacagagctgaattgtgatgattttaaaaaaggagaaagagatggggattttatctgtcctgattattatgaagctgtttgtggcacagatgggaaaacatatgacaacagatgtgcactgtgtgctgagaatgcgaaaaccgggtcccaaattggtgtaaaaagtgaaggggaatgtaagagcagtaatccagagcaggatgtatgcagtgcttttcggccctttgttagagatggaagacttggatgcacaagggaaaatgatcctgttcttggtcctgatgggaagacgcatggcaataagtgtgcaatgtgtgctgagctgtttttaaaagaagctgaaaatgccaagcgagagggtgaaactagaattcgacgaaatgctgaaaaggatttttgcaaggaatatgaaaaacaagtgagaaatggaaggcttttttgtacacgggagagtgatccagtccgtggccctgacggcaggatgcatggcaacaaatgtgccctgtgtgctgaaattttcaagcagcgtttttcagaggaaaacagtaaaacagatcaaaatttgggaaaagctgaagaaaaaactaaagttaaaagagaaattgtgaaactctgcagtcaatatcaaaatcaggcaaagaatggaatacttttctgtaccagagaaaatgaccctattcgtggtccagatgggaaaatgcatggcaacttgtgttccatgtgtcaagcctacttccaagcagaaaatgaagaaaagaaaaaggctgaagcacgagctagaaacaaaagagaatctggaaaagcaacctcatatgcagagctttgcagtgaatatcgaaagcttgtgaggaacggaaaacttgcttgcaccagagagaacgatcctatccagggcccagatgggaaagtgcatggcaacacctgctccatgtgtgaggtcttcttccaagcagaagaagaagaaaagaaaaagaaggaaggtaaatcaagaaacaaaagacaatctaagagtacagcttcctttgaggagttgtgtagtgaataccgcaaatccaggaaaaacggacggcttttttgcaccagagagaatgaccccatccagggcccagatggaaaaatgcatggcaacacctgctccatgtgtgaggccttctttcaacaagaagaaagagcaagagcaaaggctaaaagagaagctgcaaaggaaatctgcagtgaatttcgggaccaagtgaggaatggaacacttatatgcaccagggagcataatcctgtccgtggcccagatggcaaaatgcatggaaacaagtgtgccatgtgtgccagtgtgttcaaacttgaagaagaagagaagaaaaatgataaagaagaaaaagggaaagtcgaggctgaaaaagttaagagagaagcagttcaggagctgtgcagtgaatatcgtcattatgtgaggaatggacgactcccctgtaccagagagaatgatcctattgagggtctagatgggaaaatccacggcaacacctgctccatgtgtgaagccttcttccagcaagaagcaaaagaaaaagaaagagctgaacccagagcaaaagtcaaaagagaagctgaaaaggagacatgcgatgaatttcggagacttttgcaaaatggaaaacttttctgcacaagagaaaatgatcctgtgcgtggcccagatggcaagacccatggcaacaagtgtgccatgtgtaaggcagtcttccagaaagaaaatgaggaaagaaagaggaaagaagaggaagatcagagaaatgctgcaggacatggttccagtggtggtggaggaggaaacactcaggacgaatgtgctgagtatcgggaacaaatgaaaaatggaagactcagctgtactcgggagagtgatcctgtacgtgatgctgatggcaaatcgtacaacaatcagtgtaccatgtgtaaagcaaaattggaaagagaagcagagagaaaaaatgagtattctcgctccagatcaaatgggactggatcagaatcagggaaggatacatgtgatgagtttagaagccaaatgaaaaatggaaaactcatctgcactcgagaaagtgaccctgtccggggtccagatggcaagacacatggcaataagtgtactatgtgtaaggaaaaactggaaagggaagcagctgaaaaaaaaaagaaagaggatgaagacaggagcaatacaggagaaaggagcaatacaggagaaaggagcaatgacaaagaggatctgtgtcgtgaatttcgaagcatgcagagaaatggaaagcttatctgcaccagagaaaataaccctgttcgaggcccatatggcaagatgcacatcaataaatgtgctatgtgtcagagcatctttgatcgagaagctaatgaaagaaaaaagaaagatgaagagaaatcaagtagcaagccctcaaataatgcaaaggatgagtgcagtgaatttcgaaactatataaggaacaatgaactcatctgccctagagagaatgacccagtgcacggtgctgatggaaagttctatacaaacaagtgctacatgtgcagagctgtctttctaacagaagctttggaaagggcaaagcttcaagaaaagccatcccatgttagagcttctcaagaggaagacagcccagactctttcagttctctggattctgagatgtgcaaagactaccgagtattgcccaggataggttatctttgtccaaaggatttaaagcctgtctgtggtgacgatggccaaacctacaacaatccttgcatgctctgtcatgaaaacctgatacgccaaacaaatacacacatccgcagtacagggaagtgtgaggagagcagcaccccaggaaccaccgcagccagcatgcccccgtctgacgaa

SEQ ID NO: 120 - protein, 6 aa, synthetic construct
  REGION 1..6: note = Description of Artificial Sequence: Synthetic 6xHis tag
HHHHHH

SEQ ID NO: 121 - protein, 4 aa, synthetic construct
  REGION 1..4: note = Description of Artificial Sequence: Synthetic peptide
AAPF

SEQ ID NO: 122 - DNA, 21 bp, synthetic construct
  misc_feature 1..21: note = Description of Artificial Sequence: Synthetic oligonucleotide
  source 1..21: mol_type = other DNA
atgcgtcgtatgcgtcgtatg

SEQ ID NO: 123 - DNA, 18 bp, synthetic construct
  misc_feature 1..18: note = Description of Artificial Sequence: Synthetic oligonucleotide
  source 1..18: mol_type = other DNA
gtggtggtggtggtggtg

SEQ ID NO: 124 - DNA, 22 bp, synthetic construct
  misc_feature 1..22: note = Description of Artificial Sequence: Synthetic oligonucleotide
  source 1..22: mol_type = other DNA
ttgatatgcctcctaaattttt

SEQ ID NO: 125 - DNA, 21 bp, synthetic construct
  misc_feature 1..21: note = Description of Artificial Sequence: Synthetic oligonucleotide
  source 1..21: mol_type = other DNA
taggcgcgcctattctaatgc